European Patent Specification EP 3 650 045 B1, published November 13, 2024. Title: Remedy for retinal degenerative diseases caused by photoreceptor degeneration. Applicant: DAIICHI SANKYO COMPANY, LIMITED. The sequence listing filed with the application follows.

SEQUENCE LISTING (7 sequences)

SEQ ID NO: 1 - DNA, 1873 bp, Danio rerio
gcaaagcaatgtcatttaagtgagctttaatctagatcttcaccattactcacaacatatcacacctaacaatgattaattaactcaataaaagcagcacatattcctggcagagctcatcagattgaacgctagtgcatagagatcttgtccaatcatgaggccagtgtgtgccaggtttgctctttctgtttggaagtggtatcctgttaaacataagatgtttgaaacatgtcaaatctaaactccccaaatgctgccgcaaactaaactgatagagaacatgctgctgtccctgtgttattgttcagattgtgtgaatactgagattataatgagcaattaggaacatttcccctttccatcttcccatgcagtgtggatcgtagtcagactagcaagctgctaatgtgcttaaggctcatggttgtagagtaactctcctgtaatccgcaaatcctcttcataaaacccacctgtgtgaaatatgctgagccctgagcatccaggcctttcacagggccaagggtagccgtagtccccctgactccacacaatctggaacatgcacagcttaaaataagacagaccagatttctaatcactgaattcttgtgcttcaatcagatgcggtgtgtcatctttggctggttaatcatgttttttttcagaaatctggtttctttagcgtaggtggtaatgaactggactagcatccccatgaaacgcacaacctggctaaaatgttcatcttgagctctgggatagatccttctggtatagatctattatttaacctgctttattgttgcaaagcaaagggcatcggctgcgtaataacatgctggataagttgttggttcattccgctgtggcaacccttgattaataaagggactaaactaaaaagaaaatgaatgaatgaatgaatgaaagaatgaatgaatgaataaatgttccaaagcagtttgacaaataatcagaacaataacagaattgattatgtctgaaatacgctcattctactgtggcaagtttatattttgaccatatcttagtaatttcctgcagttgtctccagttatattttagaataaaattaaaaactttaaaagacggactactctcagagaatgtgtgttggacactgaggaaggtcccgcataagcgaacgcttgtagactttcagcatgcactgagcactttgtataaacccaaatcaaacaacattgctagaatctcgacaagtgaactgtttctggacatttgcagatgagcttctgctttgccttctgatggattagattattaatttaacatagtgttaaaggtgaactcagcacaagatcctcctcttttacatgctgtctttaattatacgccacacagacactctgcagtattcacactggaccttctgagtcttgatcatggaaaagttcgatatcattttccttttgaaacgcttccgctttcaatcatttcagccaaacacaactgtgatgttgctgtctgtgtgttggagaacttcatagtagaagtgtgctgttgtgtgagagaaagttcttattatctacctgctgctcaggtacaaccttaataagttgataagttgccagatatgcagtgcaatgatggctgggattattttattatctctggcctaaatagactgctgctgacagcctggaaacatcagctaatccccattgagtctctataaagcggggtgtccgatcgccccatccagtcgtagcacggtcctgcctcgtttcttcacagtcctgcccagacatctagagattaccgcagaaggggctgagcgccacatccaaccgcagccatgaacggtacagagggaccggcattctac

SEQ ID NO: 2 - DNA, 1769 bp, Danio rerio
aaccacttgttacaaccaagctctggaatagagcatatacaacaaatttcttgaaacaagtgagctacagcagcagcagaagaagagcaagaatggtgcactcacactagaccctaattaaacacacctgatcttacttattgagtccttgaaacctacaggtgaagctaggatcacacttgacttttttccccatggacttccattcatgcgcccgcaaatgcgtcagaccacaaacgcagggtcatgcgttaagtttcacaggtcgctgcagtgcaaagtttaagcttggtaaactctgacctgcgaaatcgcatccccttttcgcagcgccgtacgacagaatttcgcacacacaaactctagtgtgaccgcagcttaagtgtgttgaagcagggttggaactaaactgtgcagggttgcggcccttcaggatctaagtttgacaccccttgactatccgaaccatgcacggttcgtttgacaagtatgagtgctctaaatcaggcccaggtgcggttcagttggccggccatggcttggttggaagaggtgtgccaaagctcagttcggttgggttttggcacggtacgcttgtagtgtaagcgcagagcacgtctgtgcccataatgcctactgattaatttggccttgggttcaaggcagctgtacctagtgtgtgtacaccctaagaataagaaactgaatctacaatttacacaagatcataattgcagttagactggacagtagactagaaaaacatttatacactcacttcatcgacgtctaataatttattttattttatttttaatctcagccctttctgcagctttgtttcacatgctcaaacactagtttgaccaaagcttaaatcagttgtgttaaataagagacattcaaaataaatgtaaatgagctctccaaatcagcagacttaacattctttaaaatgattgattcaatagtgataaaaatcaggcatagccagttgtaactttagataaattacagaaaatgtcaaatacagagaaccgattcttttttatgatacatccaagcacacatttaacacaatccaggcaaaccccgaatttcacagtcacaagcactgtttgtacaagagctttgcctaaggacacacagtctctataagtccaggtcgttggtttcactcttattttaaacatgtgacatttttcctgccatcctgtcttaggctgctgtttgcttcattccatgtcacattaaattcctcagtagcaccttttacacacacagccaatcttttccagaaaattcaattgctttgaagagataatgtgtgaacaaatccatttagaaaaggaaaattaagaatttgtaaaatcatctgtaaattgttggcattcttctgtatatgaacatcacatcatttacaggtaaaggtctggtcattaattatatgacaatttactggtattattttgtgaaaggggctattttcaatgcgttcatccatccttttcatccctcaaatctctcattcacgtccccctccccatctgcacactttatctcattttccaccctgctggaatctgagcacttgtgcagttatcagggctcctgtatttaggaggctctgggtgtccatgtaggggacgaacagaaacactgcagacctttatagaagaacaattgataagagtcctcatacataaagactccattagtaagccagtgacccaggagcccagaccaacagcaaagcagacagtgaacat

SEQ ID NO: 3 - DNA, 1179 bp, Artificial
  Base sequence of NTR-NanoLuc protein coding region
atggacatcatcagcgtggctctgaagagacacagcacaaaggcatttgatgctagcaagaagctgacacctgaacaggccgagcagatcaagacactgctccagtacagccctagcagcacaaacagccagccttggcacttcatcgtggctagcacagaggaaggcaaagctagagtggctaagagcgccgctggcaactacgtgttcaacgagagaaagatgctggatgctagccacgtggtggtgttctgtgctaagaccgccatggacgatgtgtggctgaagctggtggtggatcaggaagatgctgatggcagattcgctacacctgaagctaaggctgctaacgacaagggcagaaagttcttcgccgacatgcacagaaaggatctgcacgatgatgctgagtggatggccaagcaggtgtacctgaacgtgggcaacttcctgctgggcgtggctgctctgggcctcgatgctgtgcccatcgaaggcttcgatgctgctatcctggatgccgagttcggcctgaaggagaagggctacacaagcctggtggtggtgcctgtgggccaccacagcgtggaggacttcaacgctacactgcctaagagcagactgccccagaacatcacactgacagaggtgggcggggcgggccgggtcttcacactcgaagatttcgttggggactggcgacagacagccggctacaacctggaccaagtccttgaacagggaggtgtgtccagtttgtttcagaatctcggggtgtccgtaactccgatccaaaggattgtcctgagcggtgaaaatgggctgaagatcgacatccatgtcatcatcccgtatgaaggtctgagcggcgaccaaatgggccagatcgaaaaaatttttaaggtggtgtaccctgtggatgatcatcactttaaggtgatcctgcactatggcacactggtaatcgacggggttacgccgaacatgatcgactatttcggacggccgtatgaaggcatcgccgtgttcgacggcaaaaagatcactgtaacagggaccctgtggaacggcaacaaaattatcgacgagcgcctgatcaaccccgacggctccctgctgttccgagtaaccatcaacggagtgaccggctggcggctgtgcgaacgcattctggcgtaa

SEQ ID NO: 4 - DNA, 678 bp, Artificial
  Base sequence of DsRed2 protein coding region
atggcctcctccgagaacgtcatcaccgagttcatgcgcttcaaggtgcgcatggagggcaccgtgaacggccacgagttcgagatcgagggcgagggcgagggccgcccctacgagggccacaacaccgtgaagctgaaggtgaccaagggcggccccctgcccttcgcctgggacatcctgtccccccagttccagtacggctccaaggtgtacgtgaagcaccccgccgacatccccgactacaagaagctgtccttccccgagggcttcaagtgggagcgcgtgatgaacttcgaggacggcggcgtggcgaccgtgacccaggactcctccctgcaggacggctgcttcatctacaaggtgaagttcatcggcgtgaacttcccctccgacggccccgtgatgcagaagaagaccatgggctgggaggcctccaccgagcgcctgtacccccgcgacggcgtgctgaagggcgagacccacaaggccctgaagctgaaggacggcggccactacctggtggagttcaagtccatctacatggccaagaagcccgtgcagctgcccggctactactacgtggacgccaagctggacatcacctcccacaacgaggactacaccatcgtggagcagtacgagcgcaccgagggccgccaccacctgttcctgtag

SEQ ID NO: 5 - DNA, 1389 bp, Homo sapiens
atggccagcaacagcagctcctgcccgacacctgggggcgggcacctcaatgggtacccggtgcctccctacgccttcttcttcccccctatgctgggtggactctccccgccaggcgctctgaccactctccagcaccagcttccagttagtggatatagcacaccatccccagccaccattgagacccagagcagcagttctgaagagatagtgcccagccctccctcgccaccccctctaccccgcatctacaagccttgctttgtctgtcaggacaagtcctcaggctaccactatggggtcagcgcctgtgagggctgcaagggcttcttccgccgcagcatccagaagaacatggtgtacacgtgtcaccgggacaagaactgcatcatcaacaaggtgacccggaaccgctgccagtactgccgactgcagaagtgctttgaagtgggcatgtccaaggagtctgtgagaaacgaccgaaacaagaagaagaaggaggtgcccaagcccgagtgctctgagagctacacgctgacgccggaggtgggggagctcattgagaaggtgcgcaaagcgcaccaggaaaccttccctgccctctgccagctgggcaaatacactacgaacaacagctcagaacaacgtgtctctctggacattgacctctgggacaagttcagtgaactctccaccaagtgcatcattaagactgtggagttcgccaagcagctgcccggcttcaccaccctcaccatcgccgaccagatcaccctcctcaaggctgcctgcctggacatcctgatcctgcggatctgcacgcggtacacgcccgagcaggacaccatgaccttctcggacgggctgaccctgaaccggacccagatgcacaacgctggcttcggccccctcaccgacctggtctttgccttcgccaaccagctgctgcccctggagatggatgatgcggagacggggctgctcagcgccatctgcctcatctgcggagaccgccaggacctggagcagccggaccgggtggacatgctgcaggagccgctgctggaggcgctaaaggtctacgtgcggaagcggaggcccagccgcccccacatgttccccaagatgctaatgaagattactgacctgcgaagcatcagcgccaagggggctgagcgggtgatcacgctgaagatggagatcccgggctccatgccgcctctcatccaggaaatgttggagaactcagagggcctggacactctgagcggacagccggggggtggggggcgggacgggggtggcctggcccccccgccaggcagctgtagccccagcctcagccccagctccaacagaagcagcccggccacccactccccgtga

SEQ ID NO: 6 - DNA, 1347 bp, Homo sapiens
atgtttgactgtatggatgttctgtcagtgagtcctgggcaaatcctggatttctacactgcgagtccgtcttcctgcatgctccaggagaaagctctcaaagcatgcttcagtggattgacccaaaccgaatggcagcatcggcacactgctcaatcaattgaaacacagagcaccagctctgaggaactcgtcccaagccccccatctccacttcctccccctcgagtgtacaaaccctgcttcgtctgccaggacaaatcatcagggtaccactatggggtcagcgcctgtgagggatgtaagggctttttccgcagaagtattcagaagaatatgatttacacttgtcaccgagataagaactgtgttattaataaagtcaccaggaatcgatgccaatactgtcgactccagaagtgctttgaagtgggaatgtccaaagaatctgtcaggaatgacaggaacaagaaaaagaaggagacttcgaagcaagaatgcacagagagctatgaaatgacagctgagttggacgatctcacagagaagatccgaaaagctcaccaggaaactttcccttcactctgccagctgggtaaatacaccacgaattccagtgctgaccatcgagtccgactggacctgggcctctgggacaaattcagtgaactggccaccaagtgcattattaagatcgtggagtttgctaaacgtctgcctggtttcactggcttgaccatcgcagaccaaattaccctgctgaaggccgcctgcctggacatcctgattcttagaatttgcaccaggtataccccagaacaagacaccatgactttctcagacggccttaccctaaatcgaactcagatgcacaatgctggatttggtcctctgactgaccttgtgttcacctttgccaaccagctcctgcctttggaaatggatgacacagaaacaggccttctcagtgccatctgcttaatctgtggagaccgccaggaccttgaggaaccgacaaaagtagataagctacaagaaccattgctggaagcactaaaaatttatatcagaaaaagacgacccagcaagcctcacatgtttccaaagatcttaatgaaaatcacagatctccgtagcatcagtgctaaaggtgcagagcgtgtaattaccttgaaaatggaaattcctggatcaatgccacctctcattcaagaaatgctggagaattctgaaggacatgaacccttgaccccaagttcaagtgggaacacagcagagcacagtcctagcatctcacccagctcagtggaaaacagtggggtcagtcagtcaccactcgtgcaataa

SEQ ID NO: 7 - DNA, 1365 bp, Homo sapiens
atggccaccaataaggagcgactctttgcggctggtgccctggggcctggatctggctacccaggggcaggtttccccttcgccttcccaggggcactcagggggtctccgcctttcgagatgctgagccctagcttccggggcctgggccagcctgacctccccaaggagatggcctctctgtcggtggagacacagagcaccagctcagaggagatggtgcccagctcgccctcgccccctccgcctcctcgggtctacaagccatgcttcgtgtgcaatgacaagtcctctggctaccactatggggtcagctcttgtgaaggctgcaagggcttctttcgccgaagcatccagaagaacatggtgtacacgtgtcaccgcgacaaaaactgtatcatcaacaaggtgaccaggaatcgctgccagtactgccggctacagaagtgcttcgaagtgggcatgtccaaggaagctgtgcgaaatgaccggaacaagaagaagaaagaggtgaaggaagaagggtcacctgacagctatgagctgagccctcagttagaagagctcatcaccaaggtcagcaaagcccatcaggagactttcccctcgctctgccagctgggcaagtataccacgaactccagtgcagaccaccgcgtgcagctggatctggggctgtgggacaagttcagtgagctggctaccaagtgcatcatcaagatcgtggagtttgccaagcggttgcctggctttacagggctcagcattgctgaccagatcactctgctcaaagctgcctgcctagatatcctgatgctgcgtatctgcacaaggtacaccccagagcaggacaccatgaccttctccgacgggctgaccctgaaccggacccagatgcacaatgccggcttcgggcccctcacagaccttgtctttgcctttgctgggcagctcctgcccctggagatggatgacaccgagacagggctgctcagcgccatctgcctcatctgcggagaccgcatggacctggaggagcccgaaaaagtggacaagctgcaggagccactgctggaagccctgaggctgtacgcccggcgccggcggcccagccagccctacatgttcccaaggatgctaatgaaaatcaccgacctccggggcatcagcactaagggagctgaaagggccattactctgaagatggagattccaggcccgatgcctcccttaatccgagagatgctggagaaccctgaaatgtttgaggatgactcctcgcagcctggtccccaccccaatgcctctagcgaggatgaggttcctgggggccagggcaaagggggcctgaagtccccagcctga